European Patent Application EP 4 763 868 A1, published June 24, 2026. Title: 一种重组PTH融合蛋白及其构建方法与应用. Applicant: 康众（广东）生物医药有限公司. Application WO. The sequence listing filed with the application follows.

SEQUENCE LISTING (33 sequences)

SEQ ID NO: 1 - protein, 14 aa, synthetic construct
SVSEIQLMHNLGKH

SEQ ID NO: 2 - protein, 34 aa, synthetic construct
SVSEIQLMHNLGKHLNSMERVEWLRKKLQDVHNF

SEQ ID NO: 3 - protein, 20 aa, synthetic construct
LNSMERVEWLRKKLQDVHNF

SEQ ID NO: 4 - protein, 36 aa, synthetic construct
AVSEHQLLHDKGKSIQDLRRRFFLHHLIAEIHTAEI

SEQ ID NO: 5 - protein, 22 aa, synthetic construct
IQDLRRRFFLHHLIAEIHTAEI

SEQ ID NO: 6 - protein, 119 aa, synthetic construct
EVQLVESGGGLVQAGGSLRLSCAASGNIFANNIMGWYRQPPGKEREFVAHVSHDGDSMYAVSVKGRFAISRKDATNLYLQMNSLKPEDTAIYFCRLLNIPTQGRMEGFWGQGTQVTVSS

SEQ ID NO: 7 - protein, 123 aa, synthetic construct
QVQLVESGGGLVQTGGSLRLSCAASGSTLVGHSVGFFRQAPGKEREPVVCISSTETVMYYTNSVKGRFTISRDNAKNTVWLQMDRLAPEDTAVYYCAARPQLCSALDYRYNSWGPGTQVTVSS

SEQ ID NO: 8 - protein, 11 aa, synthetic construct
GGGGSVDDDDK

SEQ ID NO: 9 - protein, 9 aa, synthetic construct
GGGGSGGGS

SEQ ID NO: 10 - protein, 10 aa, synthetic construct
GGGGSGGGGS

SEQ ID NO: 11 - DNA, 570 bp, synthetic construct
  source 1..570: mol_type = other DNA
atggaatttaaacgtaaacggcatcaccatcaccatcacggtggaggcgggagtgtagacgatgacgataagtccgtctccgagattcagctgatgcacaacctgggcaaacacctgaactccatggaacgcgtggaatggctgcgtaaaaagctgcaggatgttcataacttcggtggtggcggttccggtggcggttctcaggtgcagctggtggaaagcggcggtggcctggttcagaccggcggtagtctgcgcctgagctgcgcagcaagtggcagtaccctggtgggccatagtgtgggctttttccgtcaggcaccgggtaaagaacgtgaaccggttgtttgcattagcagtaccgaaaccgttatgtattataccaatagtgtgaaaggccgctttaccattagtcgcgataatgcaaaaaataccgtttggctgcagatggatcgcctggccccggaagataccgcagtgtattattgtgccgcacgcccgcagctgtgtagcgccttagattatcgttataatagttggggtccgggtacccaggtgaccgttagtagt

SEQ ID NO: 12 - protein, 190 aa, synthetic construct
MEFKRKRHHHHHHGGGGSVDDDDKSVSEIQLMHNLGKHLNSMERVEWLRKKLQDVHNFGGGGSGGGSQVQLVESGGGLVQTGGSLRLSCAASGSTLVGHSVGFFRQAPGKEREPVVCISSTETVMYYTNSVKGRFTISRDNAKNTVWLQMDRLAPEDTAVYYCAARPQLCSALDYRYNSWGPGTQVTVSS

SEQ ID NO: 13 - protein, 219 aa, synthetic construct
MEFKRKRHHHHHHGGGGSVDDDDKSVSEIQLMHNLGKHLNSMERVEWLRKKLQDVHNFGGGGSGGGSLNSMERVEWLRKKLQDVHNFGGGGSGGGSQVQLVESGGGLVQTGGSLRLSCAASGSTLVGHSVGFFRQAPGKEREPVVCISSTETVMYYTNSVKGRFTISRDNAKNTVWLQMDRLAPEDTAVYYCAARPQLCSALDYRYNSWGPGTQVTVSS

SEQ ID NO: 14 - DNA, 657 bp, synthetic construct
  source 1..657: mol_type = other DNA
atggaatttaaacgtaaacggcatcaccatcaccatcacggtggaggcgggagtgtagacgatgacgataagtccgtctccgagattcagctgatgcacaacctgggcaaacacctgaactccatggaacgcgtggaatggctgcgtaaaaagctgcaggatgttcataacttcggtggtggcggtagcggcggcggtagtctgaatagcatggaacgtgttgaatggctgcgcaaaaaactgcaagatgttcataattttggtggtggcggttccggtggcggttctcaggtgcagctggtggaaagcggcggtggcctggttcagaccggcggtagtctgcgcctgagctgcgcagcaagtggcagtaccctggtgggccatagtgtgggctttttccgtcaggcaccgggtaaagaacgtgaaccggttgtttgcattagcagtaccgaaaccgttatgtattataccaatagtgtgaaaggccgctttaccattagtcgcgataatgcaaaaaataccgtttggctgcagatggatcgcctggccccggaagataccgcagtgtattattgtgccgcacgcccgcagctgtgtagcgccttagattatcgttataatagttggggtccgggtacccaggtgaccgttagtagt

SEQ ID NO: 15 - protein, 219 aa, synthetic construct
MEFKRKRHHHHHHGGGGSVDDDDKSVSEIQLMHNLGKHLNSMERVEWLRKKLQDVHNFGGGGSGGGSQVQLVESGGGLVQTGGSLRLSCAASGSTLVGHSVGFFRQAPGKEREPVVCISSTETVMYYTNSVKGRFTISRDNAKNTVWLQMDRLAPEDTAVYYCAARPQLCSALDYRYNSWGPGTQVTVSSGGGGSGGGSLNSMERVEWLRKKLQDVHNF

SEQ ID NO: 16 - DNA, 657 bp, synthetic construct
  source 1..657: mol_type = other DNA
atggaatttaaacgtaaacggcatcaccatcaccatcacggtggaggcgggagtgtagacgatgacgataagtccgtctccgagattcagctgatgcacaacctgggcaaacacctgaactccatggaacgcgtggaatggctgcgtaaaaagctgcaggatgttcataacttcggtggtggcggttccggtggcggttctcaggtgcagctggtggaaagcggcggtggcctggttcagaccggcggtagtctgcgcctgagctgcgcagcaagtggcagtaccctggtgggccatagtgtgggctttttccgtcaggcaccgggtaaagaacgtgaaccggttgtttgcattagcagtaccgaaaccgttatgtattataccaatagtgtgaaaggccgctttaccattagtcgcgataatgcaaaaaataccgtttggctgcagatggatcgcctggccccggaagataccgcagtgtattattgtgccgcacgcccgcagctgtgtagcgccttagattatcgttataatagttggggtccgggtacccaggtgaccgttagtagtggtggtggcggtagcggcggcggtagtctgaatagcatggaacgtgttgaatggctgcgcaaaaaactgcaagatgttcataatttt

SEQ ID NO: 17 - protein, 221 aa, synthetic construct
MEFKRKRHHHHHHGGGGSVDDDDKSVSEIQLMHNLGKHLNSMERVEWLRKKLQDVHNFGGGGSGGGSIQDLRRRFFLHHLIAEIHTAEIGGGGSGGGSQVQLVESGGGLVQTGGSLRLSCAASGSTLVGHSVGFFRQAPGKEREPVVCISSTETVMYYTNSVKGRFTISRDNAKNTVWLQMDRLAPEDTAVYYCAARPQLCSALDYRYNSWGPGTQVTVSS

SEQ ID NO: 18 - DNA, 663 bp, synthetic construct
  source 1..663: mol_type = other DNA
atggaatttaaacgtaaacggcatcaccatcaccatcacggtggaggcgggagtgtagacgatgacgataagtccgtctccgagattcagctgatgcacaacctgggcaaacacctgaactccatggaacgcgtggaatggctgcgtaaaaagctgcaggatgttcataacttcggtggtggcggtagcggcggcggtagtattcaggatctgcgccgtcgctttttcctgcatcatctgattgcagaaattcataccgccgaaattggtggtggcggttccggtggcggttctcaggtgcagctggtggaaagcggcggtggcctggttcagaccggcggtagtctgcgcctgagctgcgcagcaagtggcagtaccctggtgggccatagtgtgggctttttccgtcaggcaccgggtaaagaacgtgaaccggttgtttgcattagcagtaccgaaaccgttatgtattataccaatagtgtgaaaggccgctttaccattagtcgcgataatgcaaaaaataccgtttggctgcagatggatcgcctggccccggaagataccgcagtgtattattgtgccgcacgcccgcagctgtgtagcgccttagattatcgttataatagttggggtccgggtacccaggtgaccgttagtagt

SEQ ID NO: 19 - protein, 221 aa, synthetic construct
MEFKRKRHHHHHHGGGGSVDDDDKSVSEIQLMHNLGKHLNSMERVEWLRKKLQDVHNFGGGGSGGGSQVQLVESGGGLVQTGGSLRLSCAASGSTLVGHSVGFFRQAPGKEREPVVCISSTETVMYYTNSVKGRFTISRDNAKNTVWLQMDRLAPEDTAVYYCAARPQLCSALDYRYNSWGPGTQVTVSSGGGGSGGGSIQDLRRRFFLHHLIAEIHTAEI

SEQ ID NO: 20 - DNA, 663 bp, synthetic construct
  source 1..663: mol_type = other DNA
atggaatttaaacgtaaacggcatcaccatcaccatcacggtggaggcgggagtgtagacgatgacgataagtccgtctccgagattcagctgatgcacaacctgggcaaacacctgaactccatggaacgcgtggaatggctgcgtaaaaagctgcaggatgttcataacttcggtggtggcggttccggtggcggttctcaggtgcagctggtggaaagcggcggtggcctggttcagaccggcggtagtctgcgcctgagctgcgcagcaagtggcagtaccctggtgggccatagtgtgggctttttccgtcaggcaccgggtaaagaacgtgaaccggttgtttgcattagcagtaccgaaaccgttatgtattataccaatagtgtgaaaggccgctttaccattagtcgcgataatgcaaaaaataccgtttggctgcagatggatcgcctggccccggaagataccgcagtgtattattgtgccgcacgcccgcagctgtgtagcgccttagattatcgttataatagttggggtccgggtacccaggtgaccgttagtagtggtggtggcggtagcggcggcggtagtattcaggatctgcgccgtcgctttttcctgcatcatctgattgcagaaattcataccgccgaaatt

SEQ ID NO: 21 - protein, 318 aa, synthetic construct
MEFKRKRHHHHHHGGGGSVDDDDKSVSEIQLMHNLGKHLNSMERVEWLRKKLQDVHNFGGGGSGGGSEVQLVESGGGLVQAGGSLRLSCAASGNIFANNIMGWYRQPPGKEREFVAHVSHDGDSMYAVSVKGRFAISRKDATNLYLQMNSLKPEDTAIYFCRLLNIPTQGRMEGFWGQGTQVTVSSGGGGSGGGSQVQLVESGGGLVQTGGSLRLSCAASGSTLVGHSVGFFRQAPGKEREPVVCISSTETVMYYTNSVKGRFTISRDNAKNTVWLQMDRLAPEDTAVYYCAARPQLCSALDYRYNSWGPGTQVTVSS

SEQ ID NO: 22 - DNA, 954 bp, synthetic construct
  source 1..954: mol_type = other DNA
atggaatttaaacgtaaacggcatcaccatcaccatcacggtggaggcgggagtgtagacgatgacgataagtccgtctccgagattcagctgatgcacaacctgggcaaacacctgaactccatggaacgcgtggaatggctgcgtaaaaagctgcaggatgttcataacttcggtggtggcggtagcggcggcggtagtgaagttcagctggttgaaagcggtggtggcctggttcaggcaggtggcagtctgcgcctgagttgtgccgcaagcggtaatatttttgcaaataatatcatgggctggtatcgccagccgccgggtaaagaacgcgaatttgtggcccatgttagccatgatggtgacagcatgtatgcagttagtgttaaaggtcgctttgcaattagccgtaaagatgccaccaatctgtatctgcagatgaatagcctgaaaccggaagataccgcaatctatttttgtcgtctgctgaatattccgacccagggccgtatggaaggtttttggggtcagggtacccaggtgaccgttagtagtggtggtggcggttccggtggcggttctcaggtgcagctggtggaaagcggcggtggcctggttcagaccggcggtagtctgcgcctgagctgcgcagcaagtggcagtaccctggtgggccatagtgtgggctttttccgtcaggcaccgggtaaagaacgtgaaccggttgtttgcattagcagtaccgaaaccgttatgtattataccaatagtgtgaaaggccgctttaccattagtcgcgataatgcaaaaaataccgtttggctgcagatggatcgcctggccccggaagataccgcagtgtattattgtgccgcacgcccgcagctgtgtagcgccttagattatcgttataatagttggggtccgggtacccaggtgaccgttagtagt

SEQ ID NO: 23 - protein, 318 aa, synthetic construct
MEFKRKRHHHHHHGGGGSVDDDDKSVSEIQLMHNLGKHLNSMERVEWLRKKLQDVHNFGGGGSGGGSQVQLVESGGGLVQTGGSLRLSCAASGSTLVGHSVGFFRQAPGKEREPVVCISSTETVMYYTNSVKGRFTISRDNAKNTVWLQMDRLAPEDTAVYYCAARPQLCSALDYRYNSWGPGTQVTVSSGGGGSGGGSEVQLVESGGGLVQAGGSLRLSCAASGNIFANNIMGWYRQPPGKEREFVAHVSHDGDSMYAVSVKGRFAISRKDATNLYLQMNSLKPEDTAIYFCRLLNIPTQGRMEGFWGQGTQVTVSS

SEQ ID NO: 24 - DNA, 954 bp, synthetic construct
  source 1..954: mol_type = other DNA
atggaatttaaacgtaaacggcatcaccatcaccatcacggtggaggcgggagtgtagacgatgacgataagtccgtctccgagattcagctgatgcacaacctgggcaaacacctgaactccatggaacgcgtggaatggctgcgtaaaaagctgcaggatgttcataacttcggtggtggcggttccggtggcggttctcaggtgcagctggtggaaagcggcggtggcctggttcagaccggcggtagtctgcgcctgagctgcgcagcaagtggcagtaccctggtgggccatagtgtgggctttttccgtcaggcaccgggtaaagaacgtgaaccggttgtttgcattagcagtaccgaaaccgttatgtattataccaatagtgtgaaaggccgctttaccattagtcgcgataatgcaaaaaataccgtttggctgcagatggatcgcctggccccggaagataccgcagtgtattattgtgccgcacgcccgcagctgtgtagcgccttagattatcgttataatagttggggtccgggtacccaggtgaccgttagtagtggtggtggcggtagcggcggcggtagtgaagttcagctggttgaaagcggtggtggcctggttcaggcaggtggcagtctgcgcctgagttgtgccgcaagcggtaatatttttgcaaataatatcatgggctggtatcgccagccgccgggtaaagaacgcgaatttgtggcccatgttagccatgatggtgacagcatgtatgcagttagtgttaaaggtcgctttgcaattagccgtaaagatgccaccaatctgtatctgcagatgaatagcctgaaaccggaagataccgcaatctatttttgtcgtctgctgaatattccgacccagggccgtatggaaggtttttggggtcagggtacccaggtgaccgttagtagt

SEQ ID NO: 25 - protein, 217 aa, synthetic construct
MEFKRKRHHHHHHGGGGSVDDDDKSVSEIQLMHNLGKHLNSMERVEWLRKKLQDVHNFGGGGSIQDLRRRFFLHHLIAEIHTAEIGGGGSGGGSQVQLVESGGGLVQTGGSLRLSCAASGSTLVGHSVGFFRQAPGKEREPVVCISSTETVMYYTNSVKGRFTISRDNAKNTVWLQMDRLAPEDTAVYYCAARPQLCSALDYRYNSWGPGTQVTVSS

SEQ ID NO: 26 - DNA, 651 bp, synthetic construct
  source 1..651: mol_type = other DNA
atggaatttaaacgtaaacggcatcaccatcaccatcacggtggaggcgggagtgtagacgatgacgataagtccgtctccgagattcagctgatgcacaacctgggcaaacacctgaactccatggaacgcgtggaatggctgcgtaaaaagctgcaggatgttcataacttcggtggtggcggtagcattcaggatctgcgccgtcgctttttcctgcatcatctgattgcagaaattcataccgccgaaattggtggtggcggttccggtggcggttctcaggtgcagctggtggaaagcggcggtggcctggttcagaccggcggtagtctgcgcctgagctgcgcagcaagtggcagtaccctggtgggccatagtgtgggctttttccgtcaggcaccgggtaaagaacgtgaaccggttgtttgcattagcagtaccgaaaccgttatgtattataccaatagtgtgaaaggccgctttaccattagtcgcgataatgcaaaaaataccgtttggctgcagatggatcgcctggccccggaagataccgcagtgtattattgtgccgcacgcccgcagctgtgtagcgccttagattatcgttataatagttggggtccgggtacccaggtgaccgttagtagt

SEQ ID NO: 27 - protein, 227 aa, synthetic construct
MEFKRKRHHHHHHGGGGSVDDDDKSVSEIQLMHNLGKHLNSMERVEWLRKKLQDVHNFGGGGSGGGGSGGGGSIQDLRRRFFLHHLIAEIHTAEIGGGGSGGGSQVQLVESGGGLVQTGGSLRLSCAASGSTLVGHSVGFFRQAPGKEREPVVCISSTETVMYYTNSVKGRFTISRDNAKNTVWLQMDRLAPEDTAVYYCAARPQLCSALDYRYNSWGPGTQVTVSS

SEQ ID NO: 28 - DNA, 681 bp, synthetic construct
  source 1..681: mol_type = other DNA
atggaatttaaacgtaaacggcatcaccatcaccatcacggtggaggcgggagtgtagacgatgacgataagtccgtctccgagattcagctgatgcacaacctgggcaaacacctgaactccatggaacgcgtggaatggctgcgtaaaaagctgcaggatgttcataacttcggcggtggtggcagtggtggcggtggcagtggcggtggtggtagtattcaggatctgcgccgtcgctttttcctgcatcatctgattgcagaaattcataccgccgaaattggtggtggcggttccggtggcggttctcaggtgcagctggtggaaagcggcggtggcctggttcagaccggcggtagtctgcgcctgagctgcgcagcaagtggcagtaccctggtgggccatagtgtgggctttttccgtcaggcaccgggtaaagaacgtgaaccggttgtttgcattagcagtaccgaaaccgttatgtattataccaatagtgtgaaaggccgctttaccattagtcgcgataatgcaaaaaataccgtttggctgcagatggatcgcctggccccggaagataccgcagtgtattattgtgccgcacgcccgcagctgtgtagcgccttagattatcgttataatagttggggtccgggtacccaggtgaccgttagtagt

SEQ ID NO: 29 - protein, 349 aa, synthetic construct
MEFKRKRHHHHHHGGGGSVDDDDKSVSEIQLMHNLGKHLNSMERVEWLRKKLQDVHNFGGGGSGGGSEVQLVESGGGLVQAGGSLRLSCAASGNIFANNIMGWYRQPPGKEREFVAHVSHDGDSMYAVSVKGRFAISRKDATNLYLQMNSLKPEDTAIYFCRLLNIPTQGRMEGFWGQGTQVTVSSGGGGSGGGSQVQLVESGGGLVQTGGSLRLSCAASGSTLVGHSVGFFRQAPGKEREPVVCISSTETVMYYTNSVKGRFTISRDNAKNTVWLQMDRLAPEDTAVYYCAARPQLCSALDYRYNSWGPGTQVTVSSGGGGSGGGSIQDLRRRFFLHHLIAEIHTAEI

SEQ ID NO: 30 - DNA, 1047 bp, synthetic construct
  source 1..1047: mol_type = other DNA
atggaatttaaacgtaaacggcatcaccatcaccatcacggtggaggcgggagtgtagacgatgacgataagtccgtctccgagattcagctgatgcacaacctgggcaaacacctgaactccatggaacgcgtggaatggctgcgtaaaaagctgcaggatgttcataacttcggtggtggcggtagcggcggcggtagtgaagttcagctggttgaaagcggtggtggcctggttcaggcaggtggcagtctgcgcctgagttgtgccgcaagcggtaatatttttgcaaataatatcatgggctggtatcgccagccgccgggtaaagaacgcgaatttgtggcccatgttagccatgatggtgacagcatgtatgcagttagtgttaaaggtcgctttgcaattagccgtaaagatgccaccaatctgtatctgcagatgaatagcctgaaaccggaagataccgcaatctatttttgtcgtctgctgaatattccgacccagggccgtatggaaggtttttggggtcagggtacccaggtgaccgttagtagtggtggtggcggttccggtggcggttctcaggtgcagctggtggaaagcggcggtggcctggttcagaccggcggtagtctgcgcctgagctgcgcagcaagtggcagtaccctggtgggccatagtgtgggctttttccgtcaggcaccgggtaaagaacgtgaaccggttgtttgcattagcagtaccgaaaccgttatgtattataccaatagtgtgaaaggccgctttaccattagtcgcgataatgcaaaaaataccgtttggctgcagatggatcgcctggccccggaagataccgcagtgtattattgtgccgcacgcccgcagctgtgtagcgccttagattatcgttataatagttggggtccgggtacccaggtgaccgttagtagtggtggtggcggtagcggcggcggtagtattcaggatctgcgccgtcgctttttcctgcatcatctgattgcagaaattcataccgccgaaatt

SEQ ID NO: 31 - protein, 349 aa, synthetic construct
MEFKRKRHHHHHHGGGGSVDDDDKSVSEIQLMHNLGKHLNSMERVEWLRKKLQDVHNFGGGGSGGGSIQDLRRRFFLHHLIAEIHTAEIGGGGSGGGSQVQLVESGGGLVQTGGSLRLSCAASGSTLVGHSVGFFRQAPGKEREPVVCISSTETVMYYTNSVKGRFTISRDNAKNTVWLQMDRLAPEDTAVYYCAARPQLCSALDYRYNSWGPGTQVTVSSGGGGSGGGSEVQLVESGGGLVQAGGSLRLSCAASGNIFANNIMGWYRQPPGKEREFVAHVSHDGDSMYAVSVKGRFAISRKDATNLYLQMNSLKPEDTAIYFCRLLNIPTQGRMEGFWGQGTQVTVSS

SEQ ID NO: 32 - DNA, 1047 bp, synthetic construct
  source 1..1047: mol_type = other DNA
atggaatttaaacgtaaacggcatcaccatcaccatcacggtggaggcgggagtgtagacgatgacgataagtccgtctccgagattcagctgatgcacaacctgggcaaacacctgaactccatggaacgcgtggaatggctgcgtaaaaagctgcaggatgttcataacttcggtggtggcggtagcggcggcggtagtattcaggatctgcgccgtcgctttttcctgcatcatctgattgcagaaattcataccgccgaaattggtggtggcggttccggtggcggttctcaggtgcagctggtggaaagcggcggtggcctggttcagaccggcggtagtctgcgcctgagctgcgcagcaagtggcagtaccctggtgggccatagtgtgggctttttccgtcaggcaccgggtaaagaacgtgaaccggttgtttgcattagcagtaccgaaaccgttatgtattataccaatagtgtgaaaggccgctttaccattagtcgcgataatgcaaaaaataccgtttggctgcagatggatcgcctggccccggaagataccgcagtgtattattgtgccgcacgcccgcagctgtgtagcgccttagattatcgttataatagttggggtccgggtacccaggtgaccgttagtagtggtggtggcggtagcggcggcggtagtgaagttcagctggttgaaagcggtggtggcctggttcaggcaggtggcagtctgcgcctgagttgtgccgcaagcggtaatatttttgcaaataatatcatgggctggtatcgccagccgccgggtaaagaacgcgaatttgtggcccatgttagccatgatggtgacagcatgtatgcagttagtgttaaaggtcgctttgcaattagccgtaaagatgccaccaatctgtatctgcagatgaatagcctgaaaccggaagataccgcaatctatttttgtcgtctgctgaatattccgacccagggccgtatggaaggtttttggggtcagggtacccaggtgaccgttagtagt

SEQ ID NO: 33 - DNA, 15 bp, synthetic construct
  source 1..15: mol_type = other DNA
ggggsggggsggggs